European Patent Application EP 4 431 525 A1, published September 18, 2024. Title: IL-2 fusion protein. Applicant: Anaveon AG. The sequence listing filed with the application follows.

SEQUENCE LISTING (164 sequences)

SEQ ID NO: 1 - protein, 451 aa, synthetic construct
EVQLVQSGAEVKKPGESLKISCKGSGYAFTNYLIEWVRQMPGKGLEWMGVINPGSGGTNYNEKFKGQVTISADKSISTAYLQWSSLKASDTAMYYCARWRGEGYYAYFDVWGQGTTVTVSSASTKGPSVFPLAPSSKSTSGGTAALGCLVKDYFPEPVTVSWNSGALTSGVHTFPAVLQSSGLYSLSSVVTVPSSSLGTQTYICNVNHKPSNTKVDKRVEPKSCDKTHTCPPCPAPELLGGPSVFLFPPKPKDTLMISRTPEVTCVVVDVSHEDPEVKFNWYVDGVEVHNAKTKPREEQYASTYRVVSVLTVLHQDWLNGKEYKCKVSNKALPAPIEKTISKAKGQPREPQVYTLPPSREEMTKNQVSLTCLVKGFYPSDIAVEWESNGQPENNYKTTPPVLDSDGSFFLYSKLTVDKSRWQQGNVFSCSVMHEALHNHYTQKSLSLSPGK

SEQ ID NO: 2 - protein, 218 aa, synthetic construct
AIRLTQSPSSFSASTGDRVTITCKASQSVDYQGDSYMNWYQQKPGKAPKLLIYAASNLESGVPSRFSGSGSGTDFTLTISSLQSEDFATYYCQQSNEDPYTFGGGTKVEIKRTVAAPSVFIFPPSDEQLKSGTASVVCLLNNFYPREAKVQWKVDNALQSGNSQESVTEQDSKDSTYSLSSTLTLSKADYEKHKVYACEVTHQGLSSPVTKSFNRGEC

SEQ ID NO: 3 - protein, 451 aa, synthetic construct
QVQLVESGGGVVQPGRSLRLSCAASGYTFSSYLIEWVRQAPGKGLEWVAVINPGSGGTNYADSVKGRFTISADKSKNTAYLQMNSLRAEDTAVYYCARWRGDGYYAYFDVWGQGTTVTVSSASTKGPSVFPLAPSSKSTSGGTAALGCLVKDYFPEPVTVSWNSGALTSGVHTFPAVLQSSGLYSLSSVVTVPSSSLGTQTYICNVNHKPSNTKVDKRVEPKSCDKTHTCPPCPAPELLGGPSVFLFPPKPKDTLMISRTPEVTCVVVDVSHEDPEVKFNWYVDGVEVHNAKTKPREEQYNSTYRVVSVLTVLHQDWLNGKEYKCKVSNKALPAPIEKTISKAKGQPREPQVYTLPPSREEMTKNQVSLTCLVKGFYPSDIAVEWESNGQPENNYKTTPPVLDSDGSFFLYSKLTVDKSRWQQGNVFSCSVMHEALHNHYTQKSLSLSPGK

SEQ ID NO: 4 - protein, 218 aa, synthetic construct
EIVLTQSPATLSVSPGERATLSCRASQSVSYDGDSYMNWYQQKPGQAPRLLIYAASNLASGIPARFSGSGSGTEFTLTISSLQSEDAAVYYCQQSNEDPYTFGGGTKVEIKRTVAAPSVFIFPPSDEQLKSGTASVVCLLNNFYPREAKVQWKVDNALQSGNSQESVTEQDSKDSTYSLSSTLTLSKADYEKHKVYACEVTHQGLSSPVTKSFNRGEC

SEQ ID NO: 5 - protein, 153 aa, Homo sapiens
MYRMQLLSCIALSLALVTNSAPTSSSTKKTQLQLEHLLLDLQMILNGINNYKNPKLTRMLTFKFYMPKKATELKHLQCLEEELKPLEEVLNLAQSKNFHLRPRDLISNINVIVLELKGSETTFMCEYADETATIVEFLNRWITFCQSIISTLT

SEQ ID NO: 6 - protein, 134 aa, synthetic construct
MAPTSSSTKKTQLQLEHLLLDLQMILNGINNYKNPKLTRMLTFKFYMPKKATELKHLQCLEEELKPLEEVLNLAQSKNFHLRPRDLISNINVIVLELKGSETTFMCEYADETATIVEFLNRWITFSQSIISTLT

SEQ ID NO: 7 - protein, 133 aa, synthetic construct
APTSSSTKKTQLQLEHLLLDLQMILNGINNYKNPKLTAMLTAKFAMPKKATELKHLQCLEEALKPLEEVLNLAQSKNFHLRPRDLISNINVIVLELKGSETTFMCEYADETATIVEFLNRWITFCQSIISTLT

SEQ ID NO: 8 - protein, 133 aa, synthetic construct
APTSSSTKKTQLQLEHLLLDLQMILNGINNYKNPKLTRMLTAKFAMPKKATELKHLQCLEEELKPLEEVLNGAQSKNFHLRPRDLISNINVIVLELKGSETTFMCEYADETATIVEFLNRWITFCQSIISTLT

SEQ ID NO: 9 - protein, 133 aa, synthetic construct
APTSSSTKKTQLQLEHLLLDLQMILNGINNYKNPKLTRMLTFKFYMPKKATELKHLQCLEEELKPLEEVLNLAQSKNFHFDPRDVVSNINVFVLELKGSETTFMCEYADETATIVEFLNRWITFCQSIISTLT

SEQ ID NO: 10 - protein, 132 aa, synthetic construct
NFHLRPRDLISNINVIVLELKGSETTFMCEYADETATIVEFLNRWITFSQSIISTLTPTSSSTKKTQLQLEHLLLDLQMILNGINNYKNPKLTRMLTFKFYMPKKATELKHLQCLEEELKPLEEVLNLAQSK

SEQ ID NO: 11 - protein, 131 aa, synthetic construct
FHLRPRDLISNINVIVLELKGSETTFMCEYADETATIVEFLNRWITFSQSIISTLTPTSSSTKKTQLQLEHLLLDLQMILNGINNYKNPKLTRMLTFKFYMPKKATELKHLQCLEEELKPLEEVLNLAQSK

SEQ ID NO: 12 - protein, 132 aa, synthetic construct
FYMPKKATELKHLQCLEEELKPLEEVLNLAQSKNFHLRPRDLISNINVIVLELKGSETTFMCEYADETATIVEFLNRWITFSQSIISTLTPTSSSTKKTQLQLEHLLLDLQMILNGINNYKNPKLTRMLTFK

SEQ ID NO: 13 - protein, 132 aa, synthetic construct
ATIVEFLNRWITFCQSIISTLTPTSSSTKKTQLQLEHLLLDLQMILNGINNYKNPKLTRMLTFKFYMPKKATELKHLQCLEEELKPLEEVLNLAQSKNFHLRPRDLISNINVIVLELKGSETTFMCEYADET

SEQ ID NO: 14-16 - skipped (3 entries)

SEQ ID NO: 17 - protein, 4 aa, synthetic construct
GGGG

SEQ ID NO: 18 - protein, 5 aa, synthetic construct
GGGGS

SEQ ID NO: 19 - protein, 6 aa, synthetic construct
GGGGSG

SEQ ID NO: 20 - protein, 7 aa, synthetic construct
GGGGSGG

SEQ ID NO: 21 - protein, 13 aa, synthetic construct
GGGGSGGGGSGGG

SEQ ID NO: 22 - protein, 14 aa, synthetic construct
GGGGSGGGGSGGGG

SEQ ID NO: 23 - protein, 19 aa, synthetic construct
GGGGSGGGGSGGGGSGGGG

SEQ ID NO: 24 - protein, 20 aa, synthetic construct
GGGGSGGGGSGGGGSGGGGS

SEQ ID NO: 25 - protein, 349 aa, synthetic construct
AIRLTQSPSSFSASTGDRVTITCKASQSVDYNFHLRPRDLISNINVIVLELKGSETTFMCEYADETATIVEFLNRWITFSQSIISTLTPTSSSTKKTQLQLEHLLLDLQMILNGINNYKNPKLTRMLTFKFYMPKKATELKHLQCLEEELKPLEEVLNLAQSKGDSYMNWYQQKPGKAPKLLIYAASNLESGVPSRFSGSGSGTDFTLTISSLQSEDFATYYCQQSNEDPYTFGGGTKVEIKRTVAAPSVFIFPPSDEQLKSGTASVVCLLNNFYPREAKVQWKVDNALQSGNSQESVTEQDSKDSTYSLSSTLTLSKADYEKHKVYACEVTHQGLSSPVTKSFNRGEC

SEQ ID NO: 26 - protein, 353 aa, synthetic construct
AIRLTQSPSSFSASTGDRVTITCKASQSVDYGGNFHLRPRDLISNINVIVLELKGSETTFMCEYADETATIVEFLNRWITFSQSIISTLTPTSSSTKKTQLQLEHLLLDLQMILNGINNYKNPKLTRMLTFKFYMPKKATELKHLQCLEEELKPLEEVLNLAQSKGGGDSYMNWYQQKPGKAPKLLIYAASNLESGVPSRFSGSGSGTDFTLTISSLQSEDFATYYCQQSNEDPYTFGGGTKVEIKRTVAAPSVFIFPPSDEQLKSGTASVVCLLNNFYPREAKVQWKVDNALQSGNSQESVTEQDSKDSTYSLSSTLTLSKADYEKHKVYACEVTHQGLSSPVTKSFNRGEC

SEQ ID NO: 27 - protein, 355 aa, synthetic construct
AIRLTQSPSSFSASTGDRVTITCKASQSVDYGGGNFHLRPRDLISNINVIVLELKGSETTFMCEYADETATIVEFLNRWITFSQSIISTLTPTSSSTKKTQLQLEHLLLDLQMILNGINNYKNPKLTRMLTFKFYMPKKATELKHLQCLEEELKPLEEVLNLAQSKGGGGDSYMNWYQQKPGKAPKLLIYAASNLESGVPSRFSGSGSGTDFTLTISSLQSEDFATYYCQQSNEDPYTFGGGTKVEIKRTVAAPSVFIFPPSDEQLKSGTASVVCLLNNFYPREAKVQWKVDNALQSGNSQESVTEQDSKDSTYSLSSTLTLSKADYEKHKVYACEVTHQGLSSPVTKSFNRGEC

SEQ ID NO: 28 - protein, 357 aa, synthetic construct
AIRLTQSPSSFSASTGDRVTITCKASQSVDYGGGGNFHLRPRDLISNINVIVLELKGSETTFMCEYADETATIVEFLNRWITFSQSIISTLTPTSSSTKKTQLQLEHLLLDLQMILNGINNYKNPKLTRMLTFKFYMPKKATELKHLQCLEEELKPLEEVLNLAQSKGGGGSDSYMNWYQQKPGKAPKLLIYAASNLESGVPSRFSGSGSGTDFTLTISSLQSEDFATYYCQQSNEDPYTFGGGTKVEIKRTVAAPSVFIFPPSDEQLKSGTASVVCLLNNFYPREAKVQWKVDNALQSGNSQESVTEQDSKDSTYSLSSTLTLSKADYEKHKVYACEVTHQGLSSPVTKSFNRGEC

SEQ ID NO: 29 - protein, 361 aa, synthetic construct
AIRLTQSPSSFSASTGDRVTITCKASQSVDYGGGGSGNFHLRPRDLISNINVIVLELKGSETTFMCEYADETATIVEFLNRWITFSQSIISTLTPTSSSTKKTQLQLEHLLLDLQMILNGINNYKNPKLTRMLTFKFYMPKKATELKHLQCLEEELKPLEEVLNLAQSKGGGGSGGDSYMNWYQQKPGKAPKLLIYAASNLESGVPSRFSGSGSGTDFTLTISSLQSEDFATYYCQQSNEDPYTFGGGTKVEIKRTVAAPSVFIFPPSDEQLKSGTASVVCLLNNFYPREAKVQWKVDNALQSGNSQESVTEQDSKDSTYSLSSTLTLSKADYEKHKVYACEVTHQGLSSPVTKSFNRGEC

SEQ ID NO: 30 - protein, 375 aa, synthetic construct
AIRLTQSPSSFSASTGDRVTITCKASQSVDYGGGGSGGGGSGGGNFHLRPRDLISNINVIVLELKGSETTFMCEYADETATIVEFLNRWITFSQSIISTLTPTSSSTKKTQLQLEHLLLDLQMILNGINNYKNPKLTRMLTFKFYMPKKATELKHLQCLEEELKPLEEVLNLAQSKGGGGSGGGGSGGGGDSYMNWYQQKPGKAPKLLIYAASNLESGVPSRFSGSGSGTDFTLTISSLQSEDFATYYCQQSNEDPYTFGGGTKVEIKRTVAAPSVFIFPPSDEQLKSGTASVVCLLNNFYPREAKVQWKVDNALQSGNSQESVTEQDSKDSTYSLSSTLTLSKADYEKHKVYACEVTHQGLSSPVTKSFNRGEC

SEQ ID NO: 31 - protein, 387 aa, synthetic construct
AIRLTQSPSSFSASTGDRVTITCKASQSVDYGGGGSGGGGSGGGGSGGGGNFHLRPRDLISNINVIVLELKGSETTFMCEYADETATIVEFLNRWITFSQSIISTLTPTSSSTKKTQLQLEHLLLDLQMILNGINNYKNPKLTRMLTFKFYMPKKATELKHLQCLEEELKPLEEVLNLAQSKGGGGSGGGGSGGGGSGGGGSDSYMNWYQQKPGKAPKLLIYAASNLESGVPSRFSGSGSGTDFTLTISSLQSEDFATYYCQQSNEDPYTFGGGTKVEIKRTVAAPSVFIFPPSDEQLKSGTASVVCLLNNFYPREAKVQWKVDNALQSGNSQESVTEQDSKDSTYSLSSTLTLSKADYEKHKVYACEVTHQGLSSPVTKSFNRGEC

SEQ ID NO: 32 - protein, 349 aa, synthetic construct
EIVLTQSPATLSVSPGERATLSCRASQSVSYNFHLRPRDLISNINVIVLELKGSETTFMCEYADETATIVEFLNRWITFSQSIISTLTPTSSSTKKTQLQLEHLLLDLQMILNGINNYKNPKLTRMLTFKFYMPKKATELKHLQCLEEELKPLEEVLNLAQSKGDSYMNWYQQKPGQAPRLLIYAASNLASGIPARFSGSGSGTEFTLTISSLQSEDAAVYYCQQSNEDPYTFGGGTKVEIKRTVAAPSVFIFPPSDEQLKSGTASVVCLLNNFYPREAKVQWKVDNALQSGNSQESVTEQDSKDSTYSLSSTLTLSKADYEKHKVYACEVTHQGLSSPVTKSFNRGEC

SEQ ID NO: 33 - protein, 353 aa, synthetic construct
EIVLTQSPATLSVSPGERATLSCRASQSVSYGGNFHLRPRDLISNINVIVLELKGSETTFMCEYADETATIVEFLNRWITFSQSIISTLTPTSSSTKKTQLQLEHLLLDLQMILNGINNYKNPKLTRMLTFKFYMPKKATELKHLQCLEEELKPLEEVLNLAQSKGGGDSYMNWYQQKPGQAPRLLIYAASNLASGIPARFSGSGSGTEFTLTISSLQSEDAAVYYCQQSNEDPYTFGGGTKVEIKRTVAAPSVFIFPPSDEQLKSGTASVVCLLNNFYPREAKVQWKVDNALQSGNSQESVTEQDSKDSTYSLSSTLTLSKADYEKHKVYACEVTHQGLSSPVTKSFNRGEC

SEQ ID NO: 34 - protein, 355 aa, synthetic construct
EIVLTQSPATLSVSPGERATLSCRASQSVSYGGGNFHLRPRDLISNINVIVLELKGSETTFMCEYADETATIVEFLNRWITFSQSIISTLTPTSSSTKKTQLQLEHLLLDLQMILNGINNYKNPKLTRMLTFKFYMPKKATELKHLQCLEEELKPLEEVLNLAQSKGGGGDSYMNWYQQKPGQAPRLLIYAASNLASGIPARFSGSGSGTEFTLTISSLQSEDAAVYYCQQSNEDPYTFGGGTKVEIKRTVAAPSVFIFPPSDEQLKSGTASVVCLLNNFYPREAKVQWKVDNALQSGNSQESVTEQDSKDSTYSLSSTLTLSKADYEKHKVYACEVTHQGLSSPVTKSFNRGEC

SEQ ID NO: 35 - protein, 361 aa, synthetic construct
EIVLTQSPATLSVSPGERATLSCRASQSVSYGGGGSGNFHLRPRDLISNINVIVLELKGSETTFMCEYADETATIVEFLNRWITFSQSIISTLTPTSSSTKKTQLQLEHLLLDLQMILNGINNYKNPKLTRMLTFKFYMPKKATELKHLQCLEEELKPLEEVLNLAQSKGGGGSGGDSYMNWYQQKPGQAPRLLIYAASNLASGIPARFSGSGSGTEFTLTISSLQSEDAAVYYCQQSNEDPYTFGGGTKVEIKRTVAAPSVFIFPPSDEQLKSGTASVVCLLNNFYPREAKVQWKVDNALQSGNSQESVTEQDSKDSTYSLSSTLTLSKADYEKHKVYACEVTHQGLSSPVTKSFNRGEC

SEQ ID NO: 36 - protein, 375 aa, synthetic construct
EIVLTQSPATLSVSPGERATLSCRASQSVSYGGGGSGGGGSGGGNFHLRPRDLISNINVIVLELKGSETTFMCEYADETATIVEFLNRWITFSQSIISTLTPTSSSTKKTQLQLEHLLLDLQMILNGINNYKNPKLTRMLTFKFYMPKKATELKHLQCLEEELKPLEEVLNLAQSKGGGGSGGGGSGGGGDSYMNWYQQKPGQAPRLLIYAASNLASGIPARFSGSGSGTEFTLTISSLQSEDAAVYYCQQSNEDPYTFGGGTKVEIKRTVAAPSVFIFPPSDEQLKSGTASVVCLLNNFYPREAKVQWKVDNALQSGNSQESVTEQDSKDSTYSLSSTLTLSKADYEKHKVYACEVTHQGLSSPVTKSFNRGEC

SEQ ID NO: 37 - protein, 347 aa, synthetic construct
DIQMTQSPSSVSASVGDRVTITCSASQGISGNFHLRPRDLISNINVIVLELKGSETTFMCEYADETATIVEFLNRWITFSQSIISTLTPTSSSTKKTQLQLEHLLLDLQMILNGINNYKNPKLTRMLTFKFYMPKKATELKHLQCLEEELKPLEEVLNLAQSKGDLNWYQQKPGKAPKLLIYHTSSLHSGVPSRFSGSGSGTDFTLTISSLQPEDFATYYCQYYSKDLLTFGGGTKLEIKRTVAAPSVFIFPPSDEQLKSGTASVVCLLNNFYPREAKVQWKVDNALQSGNSQESVTEQDSKDSTYSLSSTLTLSKADYEKHKVYACEVTHQGLSSPVTKSFNRGEC

SEQ ID NO: 38 - protein, 351 aa, synthetic construct
DIQMTQSPSSVSASVGDRVTITCSASQGISGGGNFHLRPRDLISNINVIVLELKGSETTFMCEYADETATIVEFLNRWITFSQSIISTLTPTSSSTKKTQLQLEHLLLDLQMILNGINNYKNPKLTRMLTFKFYMPKKATELKHLQCLEEELKPLEEVLNLAQSKGGGDLNWYQQKPGKAPKLLIYHTSSLHSGVPSRFSGSGSGTDFTLTISSLQPEDFATYYCQYYSKDLLTFGGGTKLEIKRTVAAPSVFIFPPSDEQLKSGTASVVCLLNNFYPREAKVQWKVDNALQSGNSQESVTEQDSKDSTYSLSSTLTLSKADYEKHKVYACEVTHQGLSSPVTKSFNRGEC

SEQ ID NO: 39 - protein, 353 aa, synthetic construct
DIQMTQSPSSVSASVGDRVTITCSASQGISGGGGNFHLRPRDLISNINVIVLELKGSETTFMCEYADETATIVEFLNRWITFSQSIISTLTPTSSSTKKTQLQLEHLLLDLQMILNGINNYKNPKLTRMLTFKFYMPKKATELKHLQCLEEELKPLEEVLNLAQSKGGGGDLNWYQQKPGKAPKLLIYHTSSLHSGVPSRFSGSGSGTDFTLTISSLQPEDFATYYCQYYSKDLLTFGGGTKLEIKRTVAAPSVFIFPPSDEQLKSGTASVVCLLNNFYPREAKVQWKVDNALQSGNSQESVTEQDSKDSTYSLSSTLTLSKADYEKHKVYACEVTHQGLSSPVTKSFNRGEC

SEQ ID NO: 40 - protein, 359 aa, synthetic construct
DIQMTQSPSSVSASVGDRVTITCSASQGISGGGGGSGNFHLRPRDLISNINVIVLELKGSETTFMCEYADETATIVEFLNRWITFSQSIISTLTPTSSSTKKTQLQLEHLLLDLQMILNGINNYKNPKLTRMLTFKFYMPKKATELKHLQCLEEELKPLEEVLNLAQSKGGGGSGGDLNWYQQKPGKAPKLLIYHTSSLHSGVPSRFSGSGSGTDFTLTISSLQPEDFATYYCQYYSKDLLTFGGGTKLEIKRTVAAPSVFIFPPSDEQLKSGTASVVCLLNNFYPREAKVQWKVDNALQSGNSQESVTEQDSKDSTYSLSSTLTLSKADYEKHKVYACEVTHQGLSSPVTKSFNRGEC

SEQ ID NO: 41 - protein, 373 aa, synthetic construct
DIQMTQSPSSVSASVGDRVTITCSASQGISGGGGGSGGGGSGGGNFHLRPRDLISNINVIVLELKGSETTFMCEYADETATIVEFLNRWITFSQSIISTLTPTSSSTKKTQLQLEHLLLDLQMILNGINNYKNPKLTRMLTFKFYMPKKATELKHLQCLEEELKPLEEVLNLAQSKGGGGSGGGGSGGGGDLNWYQQKPGKAPKLLIYHTSSLHSGVPSRFSGSGSGTDFTLTISSLQPEDFATYYCQYYSKDLLTFGGGTKLEIKRTVAAPSVFIFPPSDEQLKSGTASVVCLLNNFYPREAKVQWKVDNALQSGNSQESVTEQDSKDSTYSLSSTLTLSKADYEKHKVYACEVTHQGLSSPVTKSFNRGEC

SEQ ID NO: 42 - protein, 111 aa, synthetic construct
AIRLTQSPSSFSASTGDRVTITCKASQSVDYQGDSYMNWYQQKPGKAPKLLIYAASNLESGVPSRFSGSGSGTDFTLTISSLQSEDFATYYCQQSNEDPYTFGGGTKVEIK

SEQ ID NO: 43 - protein, 121 aa, synthetic construct
EVQLVQSGAEVKKPGESLKISCKGSGYAFTNYLIEWVRQMPGKGLEWMGVINPGSGGTNYNEKFKGQVTISADKSISTAYLQWSSLKASDTAMYYCARWRGEGYYAYFDVWGQGTTVTVSS

SEQ ID NO: 44 - protein, 121 aa, synthetic construct
QVQLVESGGGVVQPGRSLRLSCAASGYTFSSYLIEWVRQAPGKGLEWVAVINPGSGGTNYADSVKGRFTISADKSKNTAYLQMNSLRAEDTAVYYCARWRGDGYYAYFDVWGQGTTVTVSS

SEQ ID NO: 45 - protein, 117 aa, synthetic construct
EVQLVQSGAEVKKPGESLKISCKGSGYSFTNFYIHWVRQAPGQRLEWMGSIYPNYGDTAYNQKFKDRFVFSLDTSVSTAYLQISSLKAEDTAVYYCARGYSYAMDYWGQGTTVTVSS

SEQ ID NO: 46 - protein, 258 aa, synthetic construct
EVQLVQSGAEVKKPGESLKISCKGSGYAFTNYLIEWVRQMPGKGLEWMGVINPGSGGTNYNEKFKGQVTISADKSISTAYLQWSSLKASDTAMYYCARWRGEGGGFHLRPRDLISNINVIVLELKGSETTFMCEYADETATIVEFLNRWITFSQSIISTLTPTSSSTKKTQLQLEHLLLDLQMILNGINNYKNPKLTRMLTFKFYMPKKATELKHLQCLEEELKPLEEVLNLAQSKGGGGYYAYFDVWGQGTTVTVSS

SEQ ID NO: 47 - protein, 258 aa, synthetic construct
EVQLVQSGAEVKKPGESLKISCKGSGYAFTNYLIEWVRQMPGKGLEWMGVINPGGGFYMPKKATELKHLQCLEEELKPLEEVLNLAQSKNFHLRPRDLISNINVIVLELKGSETTFMCEYADETATIVEFLNRWITFCQSIISTLTPTSSSTKKTQLQLEHLLLDLQMILNGINNYKNPKLTRMLTFKGGGSGGTNYNEKFKGQVTISADKSISTAYLQWSSLKASDTAMYYCARWRGEGYYAYFDVWGQGTTVTVSS

SEQ ID NO: 48 - protein, 330 aa, synthetic construct
ASTKGPSVFPLAPSSKSTSGGTAALGCLVKDYFPEPVTVSWNSGALTSGVHTFPAVLQSSGLYSLSSVVTVPSSSLGTQTYICNVNHKPSNTKVDKRVEPKSCDKTHTCPPCPAPELLGGPSVFLFPPKPKDTLMISRTPEVTCVVVDVSHEDPEVKFNWYVDGVEVHNAKTKPREEQYASTYRVVSVLTVLHQDWLNGKEYKCKVSNKALPAPIEKTISKAKGQPREPQVYTLPPSREEMTKNQVSLTCLVKGFYPSDIAVEWESNGQPENNYKTTPPVLDSDGSFFLYSKLTVDKSRWQQGNVFSCSVMHEALHNHYTQKSLSLSPGK

SEQ ID NO: 49 - protein, 107 aa, synthetic construct [sequence omitted]

SEQ ID NO: 50 - protein, 111 aa, synthetic construct
EIVLTQSPATLSVSPGERATLSCRASQSVSYDGDSYMNWYQQKPGQAPRLLIYAASNLASGIPARFSGSGSGTEFTLTISSLQSEDAAVYYCQQSNEDPYTFGGGTKVEIK

SEQ ID NO: 51 - protein, 451 aa, synthetic construct; identical to SEQ ID NO: 1

SEQ ID NO: 52 - protein, 355 aa, synthetic construct; identical to SEQ ID NO: 27

SEQ ID NO: 53 - protein, 447 aa, synthetic construct
QVQLVQSGAEVKKPGASVKVSCKASGYTFTNFYIHWVRQAPGQGLEWMGSIYPNYGDTAYNQKFKDRVTMTTDTSTSTAYMELRSLRSDDTAVYYCARGYSYAMDYWGQGTTVTVSSASTKGPSVFPLAPSSKSTSGGTAALGCLVKDYFPEPVTVSWNSGALTSGVHTFPAVLQSSGLYSLSSVVTVPSSSLGTQTYICNVNHKPSNTKVDKKVEPKSCDKTHTCPPCPAPELLGGPSVFLFPPKPKDTLMISRTPEVTCVVVDVSHEDPEVKFNWYVDGVEVHNAKTKPREEQYNSTYRVVSVLTVLHQDWLNGKEYKCKVSNKALPAPIEKTISKAKGQPREPQVYTLPPSRDELTKNQVSLTCLVKGFYPSDIAVEWESNGQPENNYKTTPPVLDSDGSFFLYSKLTVDKSRWQQGNVFSCSVMHEALHNHYTQKSLSLSPGK

SEQ ID NO: 54 - protein, 214 aa, synthetic construct
DIQMTQSPSSVSASVGDRVTITCSASQGISGDLNWYQQKPGKAPKLLIYHTSSLHSGVPSRFSGSGSGTDFTLTISSLQPEDFATYYCQYYSKDLLTFGGGTKLEIKRTVAAPSVFIFPPSDEQLKSGTASVVCLLNNFYPREAKVQWKVDNALQSGNSQESVTEQDSKDSTYSLSSTLTLSKADYEKHKVYACEVTHQGLSSPVTKSFNRGEC

SEQ ID NO: 55 - protein, 117 aa, synthetic construct
QVQLVQSGAEVKKPGASVKVSCKASGYTFTNFYIHWVRQAPGQGLEWMGSIYPNYGDTAYNQKFKDRVTMTVDTSTSTAYMELRSLRSDDTAVYYCARGYSYAMDYWGQGTTVTVSS

SEQ ID NO: 56 - protein, 107 aa, synthetic construct
DIQMTQSPSSVSASVGDRVTITCSASQGISGDLNWYQQKPGKAPKLLIYHTSSLHSGVPSRFSGSGSGTDFTLTISSLQPEDFATYYCQYYSKDLLTFGGGTKLEIK

SEQ ID NO: 57 - protein, 117 aa, synthetic construct
QVQLVQSGAEVKKPGASVKVSCKASGYTFTNFYIHWVRQAPGQGLEWMGSIYPNYGFTAYNQKFKDRVTMTVDTSTSTAYMELRSLRSDDTAVYYCARGYSYAMDYWGQGTTVTVSS

SEQ ID NO: 58 - protein, 107 aa, synthetic construct
DIQMTQSPSSVSASVGDRVTITCSASQGIWGDLNWYQQKPGKAPKLLIYHTSQLHSDVPSRFSGSGSGTDFTLTISSLQPEDFATYYCQGYSKDLLTFGGGTKLEIK

SEQ ID NO: 59 - protein, 117 aa, synthetic construct
QVQLVQSGAEVKKPGASVKVSCKASGYTFTNFYIHWVRQAPGQGLEWMGRIYPNYGFTAYNQKFKDRVTMTVDTSTSTAYMELRSLRSDDTAVYYCARGYSYAMDYWGQGTTVTVSS

SEQ ID NO: 60 - protein, 107 aa, synthetic construct
DIQMTQSPSSVSASVGDRVTITCSASQGIYGDLNWYQQKPGKAPKLLIYHTSSLHSGVPSRFSGSGSGTDFTLTISSLQPEDFATYYCQAYSKDLLTFGGGTKLEIK

SEQ ID NO: 61 - protein, 117 aa, synthetic construct
QVQLVQSGAEVKKPGASVKVSCKASGYTFTNFYIHWVRQAPGQGLEWMGRIYPNYGITAYNQKFKDRVTMTVDTSTSTAYMELRSLRSDDTAVYYCARGYSYAMDYWGQGTTVTVSS

SEQ ID NO: 62 - protein, 107 aa, synthetic construct
DIQMTQSPSSVSASVGDRVTITCSASQGISGDLNWYQQKPGKAPKLLIYHTSQRHSDVPSRFSGSGSGTDFTLTISSLQPEDFATYYCQGYSKDLLTFGGGTKLEIK

SEQ ID NO: 63 - protein, 117 aa, synthetic construct; identical to SEQ ID NO: 61

SEQ ID NO: 64 - protein, 107 aa, synthetic construct
DIQMTQSPSSVSASVGDRVTITCSASQGISGDLNWYQQKPGKAPKLLIYHTSSRHSGVPSRFSGSGSGTDFTLTISSLQPEDFATYYCQGYSKDLLTFGGGTKLEIK

SEQ ID NO: 65 - protein, 117 aa, synthetic construct; identical to SEQ ID NO: 61

SEQ ID NO: 66 - protein, 107 aa, synthetic construct
DIQMTQSPSSVSASVGDRVTITCSASQGIYGDLNWYQQKPGKAPKLLIYHTSSRHSGVPSRFSGSGSGTDFTLTISSLQPEDFATYYCQAYSKDLLTFGGGTKLEIK

SEQ ID NO: 67 - protein, 117 aa, synthetic construct
QVQLVQSGAEVKKPGASVKVSCKASGYTFTNFYIHWVRQAPGQGLEWMGSIYPNYGITAYNQKFKDRVTMTVDTSTSTAYMELRSLRSDDTAVYYCARGYSYAMDYWGQGTTVTVSS

SEQ ID NO: 68 - protein, 107 aa, synthetic construct
DIQMTQSPSSVSASVGDRVTITCSASQGISGDLNWYQQKPGKAPKLLIYHTSQLHSDVPSRFSGSGSGTDFTLTISSLQPEDFATYYCQGYSKDLLTFGGGTKLEIK

SEQ ID NO: 69 - protein, 114 aa, synthetic construct
QVQLVQSGAEVKKPGASVKVSCKASGYDFTSHWMHWVRQAPGQGLEWMGAIDPSDSYTNYNQKFKGRVTMTTDTSTSTAYMELRSLRSDDTAVYYCARSPFDYWGQGTTVTVSS

SEQ ID NO: 70 - protein, 107 aa, synthetic construct
DIQMTQSPSSLSASVGDRVTITCKASQDVSTAVAWYQQKPGKAPKLLIYSASYRYTGVPSRFSGSGSGTDFTFTISSLQPEDIATYYCQQHYSFPFTFGQGTKLEIK

SEQ ID NO: 71 - protein, 115 aa, synthetic construct
EVQLLESGGGLVQPGGSLRLSCAASGFTFSINAMTWVRQAPGKGLEWVSTISGSGFSTYYADSLKGRFTISRDNSKNTLYLQMNSLRAEDTAVYYCAKEVYGDYWGQGTLVTVSS

SEQ ID NO: 72 - protein, 216 aa, synthetic construct
RSVLTQPPSASGTPGQRVSISCSGNSSNIGSNSVFWYQQLPGTAPKLLIYSNNQRPSGVPDRFSGSKSGTSASLAISGLRSEDEADYYCAAWDDSLSIWVFGGGTKLTVLGQPKAAPSVTLFPPSSEELQANKATLVCLISDFYPGAVTVAWKADSSPVKAGVETTTPSKQSNNKYAASSYLSLTPEQWKSHRSYSCQVTHEGSTVEKTVAPTECS

SEQ ID NO: 73 - protein, 115 aa, synthetic construct
EVQLLESGGGLVQPGGSLRLSCAASGFTFSISAMTWVRQAPGKGLEWVSTISGSGGSTYYSDSVKGRFTISRDNSKNTLYLQINSLRADDTAVYYCAKEVYGDYWGQGTLVTVSS

SEQ ID NO: 74 - protein, 110 aa, synthetic construct
QSILTQPPSASGTPGQRVTISCSGSSSNIGSNSVFWYQQLPGTAPKLLIFSNNQRPSGVPDRFSGSKSGTSASLAISGLRSEDEADYCCAAWDDSLSGWIFGGGTKLTVL

SEQ ID NO: 75 - protein, 115 aa, synthetic construct
EVQLLESGGNLVQPGGSLRLSCAASGFTFSTYAMSWVRQAPGKGLEWVSTISGTGYSTYFADSVKGRFTISRDNSKNTLFLQMNSLRAEDTAVYYCAKEVYGDYWGQGTLVTVSS

SEQ ID NO: 76 - protein, 110 aa, synthetic construct
QSVLTQPPSASGTPGQRVTISCSGRSSNIGSNSIFWYQQLPGTAPKLLIYSNNQRPSGVPDRFSGSKSGTSASLAISGLRSEDETDYYCAAWDDSLSGWVFGGGTKLTVL

SEQ ID NO: 77 - protein, 117 aa, synthetic construct
EVLLVESGGGLVQPGGSLRLSCAASGFTFSSYSMNWVRQAPGKGLEWVSFISSSSPTLYYADSVKGRFTISRDNAKNSLYLQMNSLRDEDTAVYYCARQGLTPFDYWGQGTLVTVSS

SEQ ID NO: 78 - protein, 107 aa, synthetic construct
EIVMTQSPATLSVFPGERATLSCRASQSVSSYLAWYQQKPGQAPRLLIYGASTRATGIPARVSGSGSGTEFILTISSLQSEDFAVYYCQQYNNWPYTFGQGTKLEIK

SEQ ID NO: 79 - protein, 113 aa, synthetic construct
QVQLVESGGGVGQPGRSLRLSCAASGFTFSNYGMHWVRQAPGKGLEWVAVIWYDGSKKYYADSVKGRFTISRDNSKNTLYLQMNSLRVEDTAVYYCVGNSGHWGQGTLVTVSS

SEQ ID NO: 80 - protein, 113 aa, synthetic construct
DIVMTQTPLSLPVTPGEPASISCRSSQSLLDSDDGNTYLDWYLQKPGQSPQLLIYTLSYRASGVPDRFSGSGSGTDFTLKISRVEAEDVGVYYCMQCIEFPHTFGGGTKVEIK

SEQ ID NO: 81 - protein, 117 aa, synthetic construct
EVQLVESGGGLVQPGGSLRLSCAASGFTFSSYSMNWVRQAPGKGLQWVSYITSSSNTMYYADSVKGRFTISRDNAKNSLYLQMNSLRDEDTAVYYCASIVGAPFDYWGQGTLVTVSS

SEQ ID NO: 82 - protein, 107 aa, synthetic construct
EIVMTQSPATLSVSPGERATLSCRASQSVSSSLAWYQQKPGQAPRLLIYGASTRATGIPARFSGSGSGTEFTLTISSLQSEDFAAYYCQQYNNWPFTFGPGTKVDIK

SEQ ID NO: 83 - protein, 127 aa, synthetic construct
QVQLVQSGAEVKKPGASVKVSCKASGYTFTSYFMHWVRQAPGQGLEWMGLINPDGGNTDYAQKFQGRVTMTRDTSTSTVYMELSSLRSEDTAVYYCARDGNYYDSSGYYYPDAFDIWGQGTMVTVSS

SEQ ID NO: 84 - protein, 108 aa, synthetic construct
SSELTQDPAVSVALGQTVRITCQGDSLRRFYASWYQQKPGQAPVIVIYGKDNRPSGTPDRFSGSTSGNTASLTITGAQAEDEADYYCNSRDSSGTHVVFGGGTKLTVL

SEQ ID NO: 85 - protein, 115 aa, synthetic construct; identical to SEQ ID NO: 71

SEQ ID NO: 86 - protein, 110 aa, synthetic construct
RSVLTQPPSASGTPGQRVSISCSGASSNIGSQSVFWYQQLPGTAPKLLIYSNNQRPSGVPDRFSGSKSGTSASLAISGLRSEDEADYYCAAWDDSLSIWVFGGGTKLTVL

SEQ ID NO: 87 - protein, 110 aa, synthetic construct
RSVLTQPPSASGTPGQRVSISCSGASSNIGSSSVFWYQQLPGTAPKLLIYSNNQRPSGVPDRFSGSKSGTSASLAISGLRSEDEADYYCAAWDDSLSIWVFGGGTKLTVL

SEQ ID NO: 88 - protein, 449 aa, synthetic construct
EVQLLESGGGLVQPGGSLRLSCAASGFTFSINAMTWVRQAPGKGLEWVSTISGSGFSTYYADSLKGRFTISRDNSKNTLYLQMNSLRAEDTAVYYCAKEVYGDYWGQGTLVTVSSASVAAPSVFIFPPSDEQLKSGTASVVCLLNNFYPREAKVQWKVDNALQSGNSQESVTEQDSKDSTYSLSSTLTLSKADYEKHKVYACEVTHQGLSSPVTKSFNRGECDKTHTCPPCPAPEAAGGPSVFLFPPKPKDTLMISRTPEVTCVVVDVSHEDPEVKFNWYVDGVEVHNAKTKPREEQYNSTYRVVSVLTVLHQDWLNGKEYKCKVSNKALAAPIEKTISKAKGQPREPQVYTLPPSREEMTKNQVSLTCLVKGFYPSDIAVEWESNGQPENNYKTTPPVLDSDGSFFLTSKLTVDKSRWQQGNVFSCSVMHEALHNHYTQKSLSLSPGK

SEQ ID NO: 89 - protein, 215 aa, synthetic construct
RSVLTQPPSASGTPGQRVSISCSGASSNIGSQSVFWYQQLPGTAPKLLIYSNNQRPSGVPDRFSGSKSGTSASLAISGLRSEDEADYYCAAWDDSLSIWVFGGGTKLTVLSSASTKGPSVFPLAPSSKSTSGGTAALGCLVKDYFPEPVTVSWNSGALTSGVHTFPAVLQSSGLYSLSSVVTVPSSSLGTQTYICNVNHKPSNTKVDKRVEPKSC

SEQ ID NO: 90 - protein, 451 aa, synthetic construct
EVQLVQSGAEVKKPGESLKISCKGSGYAFTNYLIEWVRQMPGKGLEWMGVINPGSGGTNYNEKFKGQVTISADKSISTAYLQWSSLKASDTAMYYCARWRGEGYYAYFDVWGQGTTVTVSSASTKGPSVFPLAPSSKSTSGGTAALGCLVKDYFPEPVTVSWNSGALTSGVHTFPAVLQSSGLYSLSSVVTVPSSSLGTQTYICNVNHKPSNTKVDKRVEPKSCDKTHTCPPCPAPEAAGGPSVFLFPPKPKDTLMISRTPEVTCVVVDVSHEDPEVKFNWYVDGVEVHNAKTKPREEQYNSTYRVVSVLTVLHQDWLNGKEYKCKVSNKALAAPIEKTISKAKGQPREPQVYTLPPSREEMTKNQVSLYCLVKGFYPSDIAVEWESNGQPENNYKTTPPVLDSDGSFFLYSKLTVDKSRWQQGNVFSCSVMHEALHNHYTQKSLSLSPGK

SEQ ID NO: 91 - protein, 110 aa, synthetic construct
RSVLTQPPSASGTPGQRVSISCSGASSNIGSNAVFWYQQLPGTAPKLLIYSNNQRPSGVPDRFSGSKSGTSASLAISGLRSEDEADYYCAAWDDSLSIWVFGGGTKLTVL

SEQ ID NO: 92 - protein, 449 aa, synthetic construct; identical to SEQ ID NO: 88

SEQ ID NO: 93 - protein, 215 aa, synthetic construct
RSVLTQPPSASGTPGQRVSISCSGASSNIGSSSVFWYQQLPGTAPKLLIYSNNQRPSGVPDRFSGSKSGTSASLAISGLRSEDEADYYCAAWDDSLSIWVFGGGTKLTVLSSASTKGPSVFPLAPSSKSTSGGTAALGCLVKDYFPEPVTVSWNSGALTSGVHTFPAVLQSSGLYSLSSVVTVPSSSLGTQTYICNVNHKPSNTKVDKRVEPKSC

SEQ ID NO: 94 - protein, 445 aa, synthetic construct
EVQLLESGGGLVQPGGSLRLSCAASGFTFSINAMTWVRQAPGKGLEWVSTISGSGFSTYYADSLKGRFTISRDNSKNTLYLQMNSLRAEDTAVYYCAKEVYGDYWGQGTLVTVSSASTKGPSVFPLAPSSKSTSGGTAALGCLVKDYFPEPVTVSWNSGALTSGVHTFPAVLQSSGLYSLSSVVTVPSSSLGTQTYICNVNHKPSNTKVDKRVEPKSCDKTHTCPPCPAPEAAGGPSVFLFPPKPKDTLMISRTPEVTCVVVDVSHEDPEVKFNWYVDGVEVHNAKTKPREEQYNSTYRVVSVLTVLHQDWLNGKEYKCKVSNKALAAPIEKTISKAKGQPREPQVYTLPPSREEMTKNQVSLTCLVKGFYPSDIAVEWESNGQPENNYKTTPPVLDSDGSFFLTSKLTVDKSRWQQGNVFSCSVMHEALHNHYTQKSLSLSPGK

SEQ ID NO: 95 - protein, 216 aa, synthetic construct
RSVLTQPPSASGTPGQRVSISCSGASSNIGSQSVFWYQQLPGTAPKLLIYSNNQRPSGVPDRFSGSKSGTSASLAISGLRSEDEADYYCAAWDDSLSIWVFGGGTKLTVLGQPKAAPSVTLFPPSSEELQANKATLVCLISDFYPGAVTVAWKADSSPVKAGVETTTPSKQSNNKYAASSYLSLTPEQWKSHRSYSCQVTHEGSTVEKTVAPTECS

SEQ ID NO: 96 - protein, 839 aa, synthetic construct
AIRLTQSPSSFSASTGDRVTITCKASQSVDYGGGNFHLRPRDLISNINVIVLELKGSETTFMCEYADETATIVEFLNRWITFSQSIISTLTPTSSSTKKTQLQLEHLLLDLQMILNGINNYKNPKLTRMLTFKFYMPKKATELKHLQCLEEELKPLEEVLNLAQSKGGGGDSYMNWYQQKPGKAPKLLIYAASNLESGVPSRFSGSGSGTDFTLTISSLQSEDFATYYCQQSNEDPYTFGGGTKVEIKGGGGSGGGGSGGGGSEVQLVQSGAEVKKPGESLKISCKGSGYAFTNYLIEWVRQMPGKGLEWMGVINPGSGGTNYNEKFKGQVTISADKSISTAYLQWSSLKASDTAMYYCARWRGEGYYAYFDVWGQGTTVTVSSGGGGSGGGGSEVQLLESGGGLVQPGGSLRLSCAASGFTFSINAMTWVRQAPGKGLEWVSTISGSGFSTYYADSLKGRFTISRDNSKNTLYLQMNSLRAEDTAVYYCAKEVYGDYWGQGTLVTVSSASTKGPSVFPLAPSSKSTSGGTAALGCLVKDYFPEPVTVSWNSGALTSGVHTFPAVLQSSGLYSLSSVVTVPSSSLGTQTYICNVNHKPSNTKVDKRVEPKSCDKTHTCPPCPAPEAAGGPSVFLFPPKPKDTLMISRTPEVTCVVVDVSHEDPEVKFNWYVDGVEVHNAKTKPREEQYNSTYRVVSVLTVLHQDWLNGKEYKCKVSNKALAAPIEKTISKAKGQPREPQVYTLPPSREEMTKNQVSLYCLVKGFYPSDIAVEWESNGQPENNYKTTPPVLDSDGSFFLYSKLTVDKSRWQQGNVFSCSVMHEALHNHYTQKSLSLSPGK

SEQ ID NO: 97 - protein, 445 aa, synthetic construct; identical to SEQ ID NO: 94

SEQ ID NO: 98 - protein, 216 aa, synthetic construct
RSVLTQPPSASGTPGQRVSISCSGASSNIGSSSVFWYQQLPGTAPKLLIYSNNQRPSGVPDRFSGSKSGTSASLAISGLRSEDEADYYCAAWDDSLSIWVFGGGTKLTVLGQPKAAPSVTLFPPSSEELQANKATLVCLISDFYPGAVTVAWKADSSPVKAGVETTTPSKQSNNKYAASSYLSLTPEQWKSHRSYSCQVTHEGSTVEKTVAPTECS

SEQ ID NO: 99 - protein, 839 aa, synthetic construct; identical to SEQ ID NO: 96

SEQ ID NO: 100 - protein, 451 aa, synthetic construct; identical to SEQ ID NO: 90

SEQ ID NO: 101 - protein, 451 aa, synthetic construct
QVQLVQSGAEVKKPGASVKVSCKASGYTFTNFYIHWVRQAPGQGLEWMGRIYPNYGITAYNQKFKDRVTMTVDTSTSTAYMELRSLRSDDTAVYYCARGYSYAMDYWGQGTTVTVSSASVAAPSVFIFPPSDEQLKSGTASVVCLLNNFYPREAKVQWKVDNALQSGNSQESVTEQDSKDSTYSLSSTLTLSKADYEKHKVYACEVTHQGLSSPVTKSFNRGECDKTHTCPPCPAPEAAGGPSVFLFPPKPKDTLMISRTPEVTCVVVDVSHEDPEVKFNWYVDGVEVHNAKTKPREEQYNSTYRVVSVLTVLHQDWLNGKEYKCKVSNKALAAPIEKTISKAKGQPREPQVYTLPPSREEMTKNQVSLTCLVKGFYPSDIAVEWESNGQPENNYKTTPPVLDSDGSFFLTSKLTVDKSRWQQGNVFSCSVMHEALHNHYTQKSLSLSPGK

SEQ ID NO: 102 - protein, 212 aa, synthetic construct
DIQMTQSPSSVSASVGDRVTITCSASQGISGDLNWYQQKPGKAPKLLIYHTSQRHSDVPSRFSGSGSGTDFTLTISSLQPEDFATYYCQGYSKDLLTFGGGTKLEIKSSASTKGPSVFPLAPSSKSTSGGTAALGCLVKDYFPEPVTVSWNSGALTSGVHTFPAVLQSSGLYSLSSVVTVPSSSLGTQTYICNVNHKPSNTKVDKRVEPKSC

SEQ ID NO: 103 - protein, 451 aa, synthetic construct
QVQLVQSGAEVKKPGASVKVSCKASGYTFTNFYIHWVRQAPGQGLEWMGSIYPNYGITAYNQKFKDRVTMTVDTSTSTAYMELRSLRSDDTAVYYCARGYSYAMDYWGQGTTVTVSSASVAAPSVFIFPPSDEQLKSGTASVVCLLNNFYPREAKVQWKVDNALQSGNSQESVTEQDSKDSTYSLSSTLTLSKADYEKHKVYACEVTHQGLSSPVTKSFNRGECDKTHTCPPCPAPEAAGGPSVFLFPPKPKDTLMISRTPEVTCVVVDVSHEDPEVKFNWYVDGVEVHNAKTKPREEQYNSTYRVVSVLTVLHQDWLNGKEYKCKVSNKALAAPIEKTISKAKGQPREPQVYTLPPSREEMTKNQVSLTCLVKGFYPSDIAVEWESNGQPENNYKTTPPVLDSDGSFFLTSKLTVDKSRWQQGNVFSCSVMHEALHNHYTQKSLSLSPGK

SEQ ID NO: 104 - protein, 212 aa, synthetic construct
DIQMTQSPSSVSASVGDRVTITCSASQGISGDLNWYQQKPGKAPKLLIYHTSQLHSDVPSRFSGSGSGTDFTLTISSLQPEDFATYYCQGYSKDLLTFGGGTKLEIKSSASTKGPSVFPLAPSSKSTSGGTAALGCLVKDYFPEPVTVSWNSGALTSGVHTFPAVLQSSGLYSLSSVVTVPSSSLGTQTYICNVNHKPSNTKVDKRVEPKSC

SEQ ID NO: 105 - protein, 447 aa, synthetic construct
QVQLVQSGAEVKKPGASVKVSCKASGYTFTNFYIHWVRQAPGQGLEWMGRIYPNYGITAYNQKFKDRVTMTVDTSTSTAYMELRSLRSDDTAVYYCARGYSYAMDYWGQGTTVTVSSASTKGPSVFPLAPSSKSTSGGTAALGCLVKDYFPEPVTVSWNSGALTSGVHTFPAVLQSSGLYSLSSVVTVPSSSLGTQTYICNVNHKPSNTKVDKRVEPKSCDKTHTCPPCPAPEAAGGPSVFLFPPKPKDTLMISRTPEVTCVVVDVSHEDPEVKFNWYVDGVEVHNAKTKPREEQYNSTYRVVSVLTVLHQDWLNGKEYKCKVSNKALAAPIEKTISKAKGQPREPQVYTLPPSREEMTKNQVSLTCLVKGFYPSDIAVEWESNGQPENNYKTTPPVLDSDGSFFLTSKLTVDKSRWQQGNVFSCSVMHEALHNHYTQKSLSLSPGK

SEQ ID NO: 106 - protein, 214 aa, synthetic construct
DIQMTQSPSSVSASVGDRVTITCSASQGISGDLNWYQQKPGKAPKLLIYHTSQRHSDVPSRFSGSGSGTDFTLTISSLQPEDFATYYCQGYSKDLLTFGGGTKLEIKRTVAAPSVFIFPPSDEQLKSGTASVVCLLNNFYPREAKVQWKVDNALQSGNSQESVTEQDSKDSTYSLSSTLTLSKADYEKHKVYACEVTHQGLSSPVTKSFNRGEC

SEQ ID NO: 107 - protein, 841 aa, synthetic construct
AIRLTQSPSSFSASTGDRVTITCKASQSVDYGGGNFHLRPRDLISNINVIVLELKGSETTFMCEYADETATIVEFLNRWITFSQSIISTLTPTSSSTKKTQLQLEHLLLDLQMILNGINNYKNPKLTRMLTFKFYMPKKATELKHLQCLEEELKPLEEVLNLAQSKGGGGDSYMNWYQQKPGKAPKLLIYAASNLESGVPSRFSGSGSGTDFTLTISSLQSEDFATYYCQQSNEDPYTFGGGTKVEIKGGGGSGGGGSGGGGSEVQLVQSGAEVKKPGESLKISCKGSGYAFTNYLIEWVRQMPGKGLEWMGVINPGSGGTNYNEKFKGQVTISADKSISTAYLQWSSLKASDTAMYYCARWRGEGYYAYFDVWGQGTTVTVSSGGGGSGGGGSQVQLVQSGAEVKKPGASVKVSCKASGYTFTNFYIHWVRQAPGQGLEWMGRIYPNYGITAYNQKFKDRVTMTVDTSTSTAYMELRSLRSDDTAVYYCARGYSYAMDYWGQGTTVTVSSASTKGPSVFPLAPSSKSTSGGTAALGCLVKDYFPEPVTVSWNSGALTSGVHTFPAVLQSSGLYSLSSVVTVPSSSLGTQTYICNVNHKPSNTKVDKRVEPKSCDKTHTCPPCPAPEAAGGPSVFLFPPKPKDTLMISRTPEVTCVVVDVSHEDPEVKFNWYVDGVEVHNAKTKPREEQYNSTYRVVSVLTVLHQDWLNGKEYKCKVSNKALAAPIEKTISKAKGQPREPQVYTLPPSREEMTKNQVSLYCLVKGFYPSDIAVEWESNGQPENNYKTTPPVLDSDGSFFLYSKLTVDKSRWQQGNVFSCSVMHEALHNHYTQKSLSLSPGK

SEQ ID NO: 108 - protein, 447 aa, synthetic construct
QVQLVQSGAEVKKPGASVKVSCKASGYTFTNFYIHWVRQAPGQGLEWMGSIYPNYGITAYNQKFKDRVTMTVDTSTSTAYMELRSLRSDDTAVYYCARGYSYAMDYWGQGTTVTVSSASTKGPSVFPLAPSSKSTSGGTAALGCLVKDYFPEPVTVSWNSGALTSGVHTFPAVLQSSGLYSLSSVVTVPSSSLGTQTYICNVNHKPSNTKVDKRVEPKSCDKTHTCPPCPAPEAAGGPSVFLFPPKPKDTLMISRTPEVTCVVVDVSHEDPEVKFNWYVDGVEVHNAKTKPREEQYNSTYRVVSVLTVLHQDWLNGKEYKCKVSNKALAAPIEKTISKAKGQPREPQVYTLPPSREEMTKNQVSLTCLVKGFYPSDIAVEWESNGQPENNYKTTPPVLDSDGSFFLTSKLTVDKSRWQQGNVFSCSVMHEALHNHYTQKSLSLSPGK

SEQ ID NO: 109 - protein, 214 aa, synthetic construct
DIQMTQSPSSVSASVGDRVTITCSASQGISGDLNWYQQKPGKAPKLLIYHTSQLHSDVPSRFSGSGSGTDFTLTISSLQPEDFATYYCQGYSKDLLTFGGGTKLEIKRTVAAPSVFIFPPSDEQLKSGTASVVCLLNNFYPREAKVQWKVDNALQSGNSQESVTEQDSKDSTYSLSSTLTLSKADYEKHKVYACEVTHQGLSSPVTKSFNRGEC

SEQ ID NO: 110 - protein, 841 aa, synthetic construct
AIRLTQSPSSFSASTGDRVTITCKASQSVDYGGGNFHLRPRDLISNINVIVLELKGSETTFMCEYADETATIVEFLNRWITFSQSIISTLTPTSSSTKKTQLQLEHLLLDLQMILNGINNYKNPKLTRMLTFKFYMPKKATELKHLQCLEEELKPLEEVLNLAQSKGGGGDSYMNWYQQKPGKAPKLLIYAASNLESGVPSRFSGSGSGTDFTLTISSLQSEDFATYYCQQSNEDPYTFGGGTKVEIKGGGGSGGGGSGGGGSEVQLVQSGAEVKKPGESLKISCKGSGYAFTNYLIEWVRQMPGKGLEWMGVINPGSGGTNYNEKFKGQVTISADKSISTAYLQWSSLKASDTAMYYCARWRGEGYYAYFDVWGQGTTVTVSSGGGGSGGGGSQVQLVQSGAEVKKPGASVKVSCKASGYTFTNFYIHWVRQAPGQGLEWMGSIYPNYGITAYNQKFKDRVTMTVDTSTSTAYMELRSLRSDDTAVYYCARGYSYAMDYWGQGTTVTVSSASTKGPSVFPLAPSSKSTSGGTAALGCLVKDYFPEPVTVSWNSGALTSGVHTFPAVLQSSGLYSLSSVVTVPSSSLGTQTYICNVNHKPSNTKVDKRVEPKSCDKTHTCPPCPAPEAAGGPSVFLFPPKPKDTLMISRTPEVTCVVVDVSHEDPEVKFNWYVDGVEVHNAKTKPREEQYNSTYRVVSVLTVLHQDWLNGKEYKCKVSNKALAAPIEKTISKAKGQPREPQVYTLPPSREEMTKNQVSLYCLVKGFYPSDIAVEWESNGQPENNYKTTPPVLDSDGSFFLYSKLTVDKSRWQQGNVFSCSVMHEALHNHYTQKSLSLSPGK

SEQ ID NO: 111 - protein, 445 aa, synthetic construct
EVQLLESGGGLVQPGGSLRLSCAASGFTFSINAMTWVRQAPGKGLEWVSTISGSGFSTYYADSLKGRFTISRDNSKNTLYLQMNSLRAEDTAVYYCAKEVYGDYWGQGTLVTVSSASTKGPSVFPLAPSSKSTSGGTAALGCLVKDYFPEPVTVSWNSGALTSGVHTFPAVLQSSGLYSLSSVVTVPSSSLGTQTYICNVNHKPSNTKVDKRVEPKSCDKTHTCPPCPAPEAAGGPSVFLFPPKPKDTLMISRTPEVTCVVVDVSHEDPEVKFNWYVDGVEVHNAKTKPREEQYNSTYRVVSVLTVLHQDWLNGKEYKCKVSNKALAAPIEKTISKAKGQPREPQVCTLPPSREEMTKNQVSLSCAVKGFYPSDIAVEWESNGQPENNYKTTPPVLDSDGSFFLVSKLTVDKSRWQQGNVFSCSVMHEALHNHYTQKSLSLSPGK

SEQ ID NO: 112 - protein, 451 aa, synthetic construct
EVQLVQSGAEVKKPGESLKISCKGSGYAFTNYLIEWVRQMPGKGLEWMGVINPGSGGTNYNEKFKGQVTISADKSISTAYLQWSSLKASDTAMYYCARWRGEGYYAYFDVWGQGTTVTVSSASTKGPSVFPLAPSSKSTSGGTAALGCLVKDYFPEPVTVSWNSGALTSGVHTFPAVLQSSGLYSLSSVVTVPSSSLGTQTYICNVNHKPSNTKVDKRVEPKSCDKTHTCPPCPAPEAAGGPSVFLFPPKPKDTLMISRTPEVTCVVVDVSHEDPEVKFNWYVDGVEVHNAKTKPREEQYNSTYRVVSVLTVLHQDWLNGKEYKCKVSNKALAAPIEKTISKAKGQPREPQVYTLPPCREEMTKNQVSLWCLVKGFYPSDIAVEWESNGQPENNYKTTPPVLDSDGSFFLYSKLTVDKSRWQQGNVFSCSVMHEALHNHYTQKSLSLSPGK

SEQ ID NO: 113 - protein, 447 aa, synthetic construct
QVQLVQSGAEVKKPGASVKVSCKASGYTFTNFYIHWVRQAPGQGLEWMGRIYPNYGITAYNQKFKDRVTMTVDTSTSTAYMELRSLRSDDTAVYYCARGYSYAMDYWGQGTTVTVSSASTKGPSVFPLAPSSKSTSGGTAALGCLVKDYFPEPVTVSWNSGALTSGVHTFPAVLQSSGLYSLSSVVTVPSSSLGTQTYICNVNHKPSNTKVDKRVEPKSCDKTHTCPPCPAPEAAGGPSVFLFPPKPKDTLMISRTPEVTCVVVDVSHEDPEVKFNWYVDGVEVHNAKTKPREEQYNSTYRVVSVLTVLHQDWLNGKEYKCKVSNKALAAPIEKTISKAKGQPREPQVCTLPPSREEMTKNQVSLSCAVKGFYPSDIAVEWESNGQPENNYKTTPPVLDSDGSFFLVSKLTVDKSRWQQGNVFSCSVMHEALHNHYTQKSLSLSPGK

SEQ ID NO: 114 - protein, 841 aa, synthetic construct
AIRLTQSPSSFSASTGDRVTITCKASQSVDYGGGNFHLRPRDLISNINVIVLELKGSETTFMCEYADETATIVEFLNRWITFSQSIISTLTPTSSSTKKTQLQLEHLLLDLQMILNGINNYKNPKLTRMLTFKFYMPKKATELKHLQCLEEELKPLEEVLNLAQSKGGGGDSYMNWYQQKPGKAPKLLIYAASNLESGVPSRFSGSGSGTDFTLTISSLQSEDFATYYCQQSNEDPYTFGGGTKVEIKGGGGSGGGGSGGGGSEVQLVQSGAEVKKPGESLKISCKGSGYAFTNYLIEWVRQMPGKGLEWMGVINPGSGGTNYNEKFKGQVTISADKSISTAYLQWSSLKASDTAMYYCARWRGEGYYAYFDVWGQGTTVTVSSGGGGSGGGGSQVQLVQSGAEVKKPGASVKVSCKASGYTFTNFYIHWVRQAPGQGLEWMGRIYPNYGITAYNQKFKDRVTMTVDTSTSTAYMELRSLRSDDTAVYYCARGYSYAMDYWGQGTTVTVSSASTKGPSVFPLAPSSKSTSGGTAALGCLVKDYFPEPVTVSWNSGALTSGVHTFPAVLQSSGLYSLSSVVTVPSSSLGTQTYICNVNHKPSNTKVDKRVEPKSCDKTHTCPPCPAPEAAGGPSVFLFPPKPKDTLMISRTPEVTCVVVDVSHEDPEVKFNWYVDGVEVHNAKTKPREEQYNSTYRVVSVLTVLHQDWLNGKEYKCKVSNKALAAPIEKTISKAKGQPREPQVYTLPPCREEMTKNQVSLWCLVKGFYPSDIAVEWESNGQPENNYKTTPPVLDSDGSFFLYSKLTVDKSRWQQGNVFSCSVMHEALHNHYTQKSLSLSPGK

SEQ ID NO: 115 - protein, 447 aa, synthetic construct
QVQLVQSGAEVKKPGASVKVSCKASGYTFTNFYIHWVRQAPGQGLEWMGSIYPNYGITAYNQKFKDRVTMTVDTSTSTAYMELRSLRSDDTAVYYCARGYSYAMDYWGQGTTVTVSSASTKGPSVFPLAPSSKSTSGGTAALGCLVKDYFPEPVTVSWNSGALTSGVHTFPAVLQSSGLYSLSSVVTVPSSSLGTQTYICNVNHKPSNTKVDKRVEPKSCDKTHTCPPCPAPEAAGGPSVFLFPPKPKDTLMISRTPEVTCVVVDVSHEDPEVKFNWYVDGVEVHNAKTKPREEQYNSTYRVVSVLTVLHQDWLNGKEYKCKVSNKALAAPIEKTISKAKGQPREPQVCTLPPSREEMTKNQVSLSCAVKGFYPSDIAVEWESNGQPENNYKTTPPVLDSDGSFFLVSKLTVDKSRWQQGNVFSCSVMHEALHNHYTQKSLSLSPGK

SEQ ID NO: 116 - protein, 841 aa, synthetic construct
AIRLTQSPSSFSASTGDRVTITCKASQSVDYGGGNFHLRPRDLISNINVIVLELKGSETTFMCEYADETATIVEFLNRWITFSQSIISTLTPTSSSTKKTQLQLEHLLLDLQMILNGINNYKNPKLTRMLTFKFYMPKKATELKHLQCLEEELKPLEEVLNLAQSKGGGGDSYMNWYQQKPGKAPKLLIYAASNLESGVPSRFSGSGSGTDFTLTISSLQSEDFATYYCQQSNEDPYTFGGGTKVEIKGGGGSGGGGSGGGGSEVQLVQSGAEVKKPGESLKISCKGSGYAFTNYLIEWVRQMPGKGLEWMGVINPGSGGTNYNEKFKGQVTISADKSISTAYLQWSSLKASDTAMYYCARWRGEGYYAYFDVWGQGTTVTVSSGGGGSGGGGSQVQLVQSGAEVKKPGASVKVSCKASGYTFTNFYIHWVRQAPGQGLEWMGSIYPNYGITAYNQKFKDRVTMTVDTSTSTAYMELRSLRSDDTAVYYCARGYSYAMDYWGQGTTVTVSSASTKGPSVFPLAPSSKSTSGGTAALGCLVKDYFPEPVTVSWNSGALTSGVHTFPAVLQSSGLYSLSSVVTVPSSSLGTQTYICNVNHKPSNTKVDKRVEPKSCDKTHTCPPCPAPEAAGGPSVFLFPPKPKDTLMISRTPEVTCVVVDVSHEDPEVKFNWYVDGVEVHNAKTKPREEQYNSTYRVVSVLTVLHQDWLNGKEYKCKVSNKALAAPIEKTISKAKGQPREPQVYTLPPCREEMTKNQVSLWCLVKGFYPSDIAVEWESNGQPENNYKTTPPVLDSDGSFFLYSKLTVDKSRWQQGNVFSCSVMHEALHNHYTQKSLSLSPGK

SEQ ID NO: 117 - protein, 451 aa, synthetic construct
QVQLVQSGAEVKKPGASVKVSCKASGYTFTNFYIHWVRQAPGQGLEWMGSIYPNYGITAYNQKFKDRVTMTVDTSTSTAYMELRSLRSDDTAVYYCARGYSYAMDYWGQGTTVTVSSASVAAPSVFIFPPSDEQLKSGTASVVCLLNNFYPREAKVQWKVDNALQSGNSQESVTEQDSKDSTYSLSSTLTLSKADYEKHKVYACEVTHQGLSSPVTKSFNRGECDKTHTCPPCPAPEAAGGPSVFLFPPKPKDTLMISRTPEVTCVVVDVSHEDPEVKFNWYVDGVEVHNAKTKPREEQYNSTYRVVSVLTVLHQDWLNGKEYKCKVSNKALAAPIEKTISKAKGQPREPQVCTLPPSREEMTKNQVSLSCAVKGFYPSDIAVEWESNGQPENNYKTTPPVLDSDGSFFLVSKLTVDKSRWQQGNVFSCSVMHEALHNHYTQKSLSLSPGK

SEQ ID NO: 118 - protein, 10 aa, unidentified
GFTFSINAMT

SEQ ID NO: 119 - protein, 18 aa, unidentified
TISGSGFSTYYADSLKGR

SEQ ID NO: 120 - protein, 6 aa, unidentified
EVYGDY

SEQ ID NO: 121 - protein, 13 aa, unidentified
  VARIANT 3: note = X is N, S, Q, or A
  VARIANT 10..11: note = XX is NS, QS, SS, or NA
SGXSSNIGSXXVF

SEQ ID NO: 122 - protein, 7 aa, unidentified
SNNQRPS

SEQ ID NO: 123 - protein, 12 aa, unidentified
AAWDDSLSIWVF

SEQ ID NO: 124 - protein, 13 aa, unidentified
SGASSNIGSQSVF

SEQ ID NO: 125 - protein, 13 aa, unidentified
SGASSNIGSSSVF

SEQ ID NO: 126 - protein, 13 aa, unidentified
SGASSNIGSNAVF

SEQ ID NO: 127 - protein, 5 aa, unidentified
NFYIH

SEQ ID NO: 128 - protein, 17 aa, unidentified
RIYPNYGITAYNQKFKD

SEQ ID NO: 129 - protein, 8 aa, unidentified
GYSYAMDY

SEQ ID NO: 130 - protein, 11 aa, unidentified
SASQGISGDLN

SEQ ID NO: 131 - protein, 7 aa, unidentified
HTSQRHS

SEQ ID NO: 132 - protein, 9 aa, unidentified
QGYSKDLLT

SEQ ID NO: 133 - protein, 17 aa, unidentified
SIYPNYGITAYNQKFKD

SEQ ID NO: 134 - protein, 7 aa, unidentified
HTSQLHS

SEQ ID NO: 135 - protein, 10 aa, unidentified
GFTFSISAMT

SEQ ID NO: 136 - protein, 17 aa, unidentified
TISGSGGSTYYSDSVKG

SEQ ID NO: 137 - protein, 11 aa, unidentified
SGSSSNIGSNS

SEQ ID NO: 138 - protein, 10 aa, unidentified
GFTFSTYAMS

SEQ ID NO: 139 - protein, 17 aa, unidentified
TISGTGYSTYFADSVKG

SEQ ID NO: 140 - protein, 11 aa, unidentified
SGRSSNIGSNS

SEQ ID NO: 141 - protein, 11 aa, unidentified
AAWDDSLSGWV

SEQ ID NO: 142 - protein, 8 aa, unidentified
GFTFSSYS

SEQ ID NO: 143 - protein, 17 aa, unidentified
FISSSSPTLYYADSVKG

SEQ ID NO: 144 - protein, 10 aa, unidentified
ARQGLTPFDY

SEQ ID NO: 145 - protein, 11 aa, unidentified
RASQSVSSYLA

SEQ ID NO: 146 - protein, 7 aa, unidentified
GASTRAT

SEQ ID NO: 147 - protein, 9 aa, unidentified
QQYNNWPYT

SEQ ID NO: 148 - protein, 10 aa, unidentified
GFTFSNYGMH

SEQ ID NO: 149 - protein, 17 aa, unidentified
VIWYDGSKKYYADSVKG

SEQ ID NO: 150 - protein, 4 aa, unidentified
NSGH

SEQ ID NO: 151 - protein, 17 aa, unidentified
RSSQSLLDSDDGNTYLD

SEQ ID NO: 152 - protein, 7 aa, unidentified
TLSYRAS

SEQ ID NO: 153 - protein, 9 aa, unidentified
MQCIEFPHT

SEQ ID NO: 154 - protein, 10 aa, unidentified
GFTFSSYSMN

SEQ ID NO: 155 - protein, 17 aa, unidentified
YITSSSNTMYYADSVKG

SEQ ID NO: 156 - protein, 8 aa, unidentified
IVGAPFDY

SEQ ID NO: 157 - protein, 11 aa, unidentified
RASQSVSSSLA

SEQ ID NO: 158 - protein, 9 aa, unidentified
QQYNNWPFT

SEQ ID NO: 159 - protein, 10 aa, unidentified
GYTFTSYFMH

SEQ ID NO: 160 - protein, 17 aa, unidentified
LINPDGGNTDYAQKFQG

SEQ ID NO: 161 - protein, 18 aa, unidentified
DGNYYDSSGYYYPDAFDI

SEQ ID NO: 162 - protein, 11 aa, unidentified
QGDSLRRFYAS

SEQ ID NO: 163 - protein, 7 aa, unidentified
GKDNRPS

SEQ ID NO: 164 - protein, 11 aa, unidentified
NSRDSSGTHVV